European Patent Application EP 4 180 446 A1, published May 17, 2023. Title: Cyclic Peptide, Peptide Complex and Pharmaceutical Composition. Applicant: The University of Tokyo. The sequence listing filed with the application follows.

SEQUENCE LISTING (22 sequences)

SEQ ID NO: 1 - protein, 19 aa, Artificial Sequence
  partial structure of cyclic peptide isolated from L-peptide library based on RaPID system, TrbL1
YRHNSYEASAFWCGSGSGS

SEQ ID NO: 2 - protein, 19 aa, Artificial Sequence
  partial structure of cyclic peptide isolated from L-peptide library based on RaPID system
YRHNSYKASAFWCGSGSGS

SEQ ID NO: 3 - protein, 19 aa, Artificial Sequence
  partial structure of cyclic peptide isolated from L-peptide library based on RaPID system
YRHSSYEASAFWCGSGSGS

SEQ ID NO: 4 - protein, 19 aa, Artificial Sequence
  partial structure of cyclic peptide isolated from L-peptide library based on RaPID system
YRHDSYEASAFWCGSGSGS

SEQ ID NO: 5 - protein, 19 aa, Artificial Sequence
  partial structure of cyclic peptide isolated from L-peptide library based on RaPID system
YRHNSYEASTFWCGSGSGS

SEQ ID NO: 6 - protein, 19 aa, Artificial Sequence
  partial structure of cyclic peptide isolated from L-peptide library based on RaPID system
YRHNSYEASAFCCGSGSGS

SEQ ID NO: 7 - protein, 16 aa, Artificial Sequence
  partial structure of cyclic peptide isolated from L-peptide library based on RaPID system, TrbL3
YLRPRYKFWCGSGSGS

SEQ ID NO: 8 - protein, 16 aa, Artificial Sequence
  partial structure of cyclic peptide isolated from L-peptide library based on RaPID system
YLQPKFKFWCGSGSGS

SEQ ID NO: 9 - protein, 19 aa, Artificial Sequence
  partial structure of cyclic peptide isolated from L-peptide library based on RaPID system
YAHEGYKNSAFWCGSGSGS

SEQ ID NO: 10 - protein, 18 aa, Artificial Sequence
  partial structure of cyclic peptide isolated from L-peptide library based on RaPID system, TrbL2
YRFWQTPRFRLCGSGSGS

SEQ ID NO: 11 - protein, 19 aa, Artificial Sequence
  partial structure of cyclic peptide isolated from L-peptide library based on RaPID system
YKYKFWAYIPTNCGSGSGS

SEQ ID NO: 12 - protein, 18 aa, Artificial Sequence
  partial structure of cyclic peptide isolated from L-peptide library based on RaPID system
YRIHPWITTYRCGSGSGS

SEQ ID NO: 13 - protein, 18 aa, Artificial Sequence
  partial structure of cyclic peptide isolated from L-peptide library based on RaPID system
YRLHQWINTFRCGSGSGS

SEQ ID NO: 14 - DNA, 29 bp, Artificial Sequence
  Designed oligonucleotide primer for PCR
acggaagctcactcaggcatgcatgcctt

SEQ ID NO: 15 - DNA, 30 bp, Artificial Sequence
  Designed oligonucleotide primer for PCR
catgaggtccccccaccctgtttgctgctg

SEQ ID NO: 16 - DNA, 25 bp, Artificial Sequence
  Designed oligonucleotide primer for PCR
agttttctctactactactacatcc

SEQ ID NO: 17 - DNA, 29 bp, Artificial Sequence
  Designed oligonucleotide primer for PCR
aaaagttggcactagacgacgacgacgac

SEQ ID NO: 18 - DNA, 20 bp, Artificial Sequence
  Designed oligonucleotide primer for PCR
ggtgagctgactgaccaaat

SEQ ID NO: 19 - DNA, 32 bp, Artificial Sequence
  Designed oligonucleotide primer for PCR
ttcactggtatcatcactgatcactgctgctg

SEQ ID NO: 20 - protein, 13 aa, Artificial Sequence
  partial structure of cyclic peptide
YRHNSYEASAFWC

SEQ ID NO: 21 - protein, 12 aa, Artificial Sequence
  partial structure of cyclic peptide
YRFWQTPRFRLC

SEQ ID NO: 22 - protein, 10 aa, Artificial Sequence
  partial structure of cyclic peptide
YLRPRYKFWC